European Patent Application EP 4 775 221 A1, published July 15, 2026. Title: Composition for preventing from Mycoplasma hyorhinis infection and the production method thereof. Applicant: 财团法人农业科技研究院. Application CN. The sequence listing filed with the application follows.

SEQUENCE LISTING (13 sequences)

SEQ ID NO: 1 - DNA, 60 bp, synthetic construct
  source 1..60: mol_type = other DNA
atatacatatgagaggatcgcaccaccaccaccaccacccgattatggatgcgctgaaag

SEQ ID NO: 2 - DNA, 33 bp, synthetic construct
  source 1..33: mol_type = other DNA
caatatgtcgacttaatgatgatgatgatgatg

SEQ ID NO: 3 - DNA, 23 bp, synthetic construct
  source 1..23: mol_type = other DNA
cactataggggaattgtgagcgg

SEQ ID NO: 4 - DNA, 22 bp, synthetic construct
  source 1..22: mol_type = other DNA
gctagttattgctcagcggtgg

SEQ ID NO: 5 - DNA, 8322 bp, synthetic construct
  source 1..8322: mol_type = other DNA
atccggatatagttcctcctttcagcaaaaaacccctcaagacccgtttagaggccccaaggggttatgctagttattgctcagcggtggcagcagccaactcagcttcctttcgggctttgttagcagccggatctcagtggtggtggtggtggtgctcgagtgcggccgcaagcttgtcgacttaatgatgatgatgatgatgctgggtcacgccattggtcggaacggtgccgctcgcgctaacgctaacattcgcgctggtgctttgctgcgcgttcgccagcgggttgtcaacgttctgcttggtcacaaccaccgggttcaccagaatcgccttgatgtttttgtacgcgccaacgctacccgctttgtaggtggtatcgtcataacggaagtggatatccttggtgttttcgttgtttttcagcgcgttctccacgtcttctttggtcgcggtcgcgttcgctttctttttgttaatcagggttttcagaacttccaccgcaaccttgcccaggataacgtccggtttgtaaatggtcatgttctgctcgccgttcttgatcagctttttcgcggtgtcgttgtaatcctgaccggtgatgaaaaccttttgcacatcgtagttggtcgctttcagcttgtcaaccgcctgctccgccataccatcgttcggcgccaggaaacccttcagaacgcttttcgggatggtcacgttatcgtaggtaaccggcagcacaccgttcggcacgctgctgtcacgatattgggtaaagaattgctgaatacgctggcccgcatcaccgtagttccagcccggcacataaaccgcgttaccacgcgggctcaggtcaaccactttgccgttgctgttttccatcagctttttcaggatcttcatcgcgccgttataaaagtactggctgttgttatcgtcttggctacccgcaaccgcgtagaagctcacggtttcttgcggcatgtgatccttcagatagttcagcatctcggtttcgtccttaaacgcaccatcggttttacccagcagacccgccgccaggctcaggccttgcagctcgccaaccttttcgttgtcgtagctaacgtaccaatcgtagctggtgctgccggtgatcagacggtcgtacgccacaatcgggatgttcttctccgcaatgctgttaaccgcggtgcccacgccaccgccgttctccggcgcaatgatgaaacccttcggcgccgggttcaggttcgcttgctgggtcagccagttgttctgcgcgttttgatctttggtaatggtgctgatcgcaccttcggtcttgtcgatgtagttcaggatatccttttgcgcgttgatccaacgcgggttatccgggtcggtcagcgcaacacgaatgctctcgttggtcaccgcgtggtctttggtctggctcaggccggtcgcggtggtgccgcacgcaacaaagctggatcccttcgcagccgcttctttagcagccgcctctttagcagcagcctcatctttcacatctttgctcagcttggtggtgtcgatttcggtgttatcgtaaatcttctgcgcaaactcgaacgcctttttgatgtcgctaaaggtgctatcgttaacggtatagccgctgaaaccggtgtttttgctgctttctttaatcttgatcgcgctgaacatgctgctgctcgggatgtggttgcctttaccctccgcttccttcacctttttcgcaatgatgctgttctcgtcaatggtgccaccaccctgcttgatgatgtcgaacagaaccttcatgatatccaggttgaacacaataccatcggtgtcgttgatgttgtacggcaggctcttcagggtggtctggccctcaacacccagcagcttgttatagttgttaatgattttggtcggaaagctgttcgggttaacggtgctggtgcccacgtccagcagtttatcgtagctgttcgccacatacgcggtcgccttgttgcccaggatcaggttccaatcgctgctttgcttggtgctcagatcgctgtccaggctgctcagcagctgaccctcgctgtttttgtgggtaacgtcgctggtcagcagctccaccgggataaaatccgcgtcgtttttatgctgttcgttgtaaatcttgatgatctccttcatgcccagcatcatcggccaatagctaccttggctggtcgcgaacttgatggtggtcggctgaccggtacctttcgccgccgcctctttcgccgccgcttctttcgccgccgcctcgttttctttcacttccgcttcaatcggttgatcgtcgctgctggtgtcgctggtgttcgcttgctgcgccgccgcctgcgcaaacgcctgcgccgcttgttcgatctgatccagtttggtcttcagctcttcaattttctcttccttaaccaggtccttcagctcttggatctgtttctccagggtttctttttgcttcgcgtccactttatcaccctggtcctccaggctcttttccagttggttgatcagcgcttccgcacgcacggtaacctcaatcttttcctttttcttcgcatccgcctcacggttctcttccgcctctttcaccatacgttcgatctcttcctcgctcaggctggtggtgttcttaatggtgatggtctgttccttgttggttttcttatctttcgcgctaacggtggtaatgccgttcacgtcgatgctaaagctaacttcgatctgcggcacaccacgcggcgcttgctcaatgccgctcaggttgaaacgacccagcagcttgttgtccgccgccagctgacgctcgccttgaaccacgctgatggtaacctcggtttggttgttttccgcggtgctgaaaatctggcttttggtcaccggaatggtggtgttacgcggaatcagcggggtcgcaatgccacccagggtttcgatacccagggtcagcggggtaacgtccagcagcagcacatcgttaatctcgcccgccagaacgccaccttgaatcgccgcaccgatcgcaaccacttcgtccgggttaatgctacggttcggtttcttgcccagggtgtgctcaatcatggtctgcaccgccggaatacgggtgctaccgccaaccagcagaacttcgtccaggtccttcgcctccagcttcgcctctttcagcgcatccataatcgggtggtggtggtggtggtgcgatcctctcatatgtatatctccttcttaaagttaaacaaaattatttctagaggggaattgttatccgctcacaattcccctatagtgagtcgtattaatttcgcgggatcgagatcgatctcgatcctctacgccggacgcatcgtggccggcatcaccggcgccacaggtgcggttgctggcgcctatatcgccgacatcaccgatggggaagatcgggctcgccacttcgggctcatgagcgcttgtttcggcgtgggtatggtggcaggccccgtggccgggggactgttgggcgccatctccttgcatgcaccattccttgcggcggcggtgctcaacggcctcaacctactactgggctgcttcctaatgcaggagtcgcataagggagagcgtcgagatcccggacaccatcgaatggcgcaaaacctttcgcggtatggcatgatagcgcccggaagagagtcaattcagggtggtgaatgtgaaaccagtaacgttatacgatgtcgcagagtatgccggtgtctcttatcagaccgtttcccgcgtggtgaaccaggccagccacgtttctgcgaaaacgcgggaaaaagtggaagcggcgatggcggagctgaattacattcccaaccgcgtggcacaacaactggcgggcaaacagtcgttgctgattggcgttgccacctccagtctggccctgcacgcgccgtcgcaaattgtcgcggcgattaaatctcgcgccgatcaactgggtgccagcgtggtggtgtcgatggtagaacgaagcggcgtcgaagcctgtaaagcggcggtgcacaatcttctcgcgcaacgcgtcagtgggctgatcattaactatccgctggatgaccaggatgccattgctgtggaagctgcctgcactaatgttccggcgttatttcttgatgtctctgaccagacacccatcaacagtattattttctcccatgaagacggtacgcgactgggcgtggagcatctggtcgcattgggtcaccagcaaatcgcgctgttagcgggcccattaagttctgtctcggcgcgtctgcgtctggctggctggcataaatatctcactcgcaatcaaattcagccgatagcggaacgggaaggcgactggagtgccatgtccggttttcaacaaaccatgcaaatgctgaatgagggcatcgttcccactgcgatgctggttgccaacgatcagatggcgctgggcgcaatgcgcgccattaccgagtccgggctgcgcgttggtgcggacatctcggtagtgggatacgacgataccgaagacagctcatgttatatcccgccgttaaccaccatcaaacaggattttcgcctgctggggcaaaccagcgtggaccgcttgctgcaactctctcagggccaggcggtgaagggcaatcagctgttgcccgtctcactggtgaaaagaaaaaccaccctggcgcccaatacgcaaaccgcctctccccgcgcgttggccgattcattaatgcagctggcacgacaggtttcccgactggaaagcgggcagtgagcgcaacgcaattaatgtaagttagctcactcattaggcaccgggatctcgaccgatgcccttgagagccttcaacccagtcagctccttccggtgggcgcggggcatgactatcgtcgccgcacttatgactgtcttctttatcatgcaactcgtaggacaggtgccggcagcgctctgggtcattttcggcgaggaccgctttcgctggagcgcgacgatgatcggcctgtcgcttgcggtattcggaatcttgcacgccctcgctcaagccttcgtcactggtcccgccaccaaacgtttcggcgagaagcaggccattatcgccggcatggcggccccacgggtgcgcatgatcgtgctcctgtcgttgaggacccggctaggctggcggggttgccttactggttagcagaatgaatcaccgatacgcgagcgaacgtgaagcgactgctgctgcaaaacgtctgcgacctgagcaacaacatgaatggtcttcggtttccgtgtttcgtaaagtctggaaacgcggaagtcagcgccctgcaccattatgttccggatctgcatcgcaggatgctgctggctaccctgtggaacacctacatctgtattaacgaagcgctggcattgaccctgagtgatttttctctggtcccgccgcatccataccgccagttgtttaccctcacaacgttccagtaaccgggcatgttcatcatcagtaacccgtatcgtgagcatcctctctcgtttcatcggtatcattacccccatgaacagaaatcccccttacacggaggcatcagtgaccaaacaggaaaaaaccgcccttaacatggcccgctttatcagaagccagacattaacgcttctggagaaactcaacgagctggacgcggatgaacaggcagacatctgtgaatcgcttcacgaccacgctgatgagctttaccgcagctgcctcgcgcgtttcggtgatgacggtgaaaacctctgacacatgcagctcccggagacggtcacagcttgtctgtaagcggatgccgggagcagacaagcccgtcagggcgcgtcagcgggtgttggcgggtgtcggggcgcagccatgacccagtcacgtagcgatagcggagtgtatactggcttaactatgcggcatcagagcagattgtactgagagtgcaccatatatgcggtgtgaaataccgcacagatgcgtaaggagaaaataccgcatcaggcgctcttccgcttcctcgctcactgactcgctgcgctcggtcgttcggctgcggcgagcggtatcagctcactcaaaggcggtaatacggttatccacagaatcaggggataacgcaggaaagaacatgtgagcaaaaggccagcaaaaggccaggaaccgtaaaaaggccgcgttgctggcgtttttccataggctccgcccccctgacgagcatcacaaaaatcgacgctcaagtcagaggtggcgaaacccgacaggactataaagataccaggcgtttccccctggaagctccctcgtgcgctctcctgttccgaccctgccgcttaccggatacctgtccgcctttctcccttcgggaagcgtggcgctttctcatagctcacgctgtaggtatctcagttcggtgtaggtcgttcgctccaagctgggctgtgtgcacgaaccccccgttcagcccgaccgctgcgccttatccggtaactatcgtcttgagtccaacccggtaagacacgacttatcgccactggcagcagccactggtaacaggattagcagagcgaggtatgtaggcggtgctacagagttcttgaagtggtggcctaactacggctacactagaaggacagtatttggtatctgcgctctgctgaagccagttaccttcggaaaaagagttggtagctcttgatccggcaaacaaaccaccgctggtagcggtggtttttttgtttgcaagcagcagattacgcgcagaaaaaaaggatctcaagaagatcctttgatcttttctacggggtctgacgctcagtggaacgaaaactcacgttaagggattttggtcatgaacaataaaactgtctgcttacataaacagtaatacaaggggtgttatgagccatattcaacgggaaacgtcttgctctaggccgcgattaaattccaacatggatgctgatttatatgggtataaatgggctcgcgataatgtcgggcaatcaggtgcgacaatctatcgattgtatgggaagcccgatgcgccagagttgtttctgaaacatggcaaaggtagcgttgccaatgatgttacagatgagatggtcagactaaactggctgacggaatttatgcctcttccgaccatcaagcattttatccgtactcctgatgatgcatggttactcaccactgcgatccccgggaaaacagcattccaggtattagaagaatatcctgattcaggtgaaaatattgttgatgcgctggcagtgttcctgcgccggttgcattcgattcctgtttgtaattgtccttttaacagcgatcgcgtatttcgtctcgctcaggcgcaatcacgaatgaataacggtttggttgatgcgagtgattttgatgacgagcgtaatggctggcctgttgaacaagtctggaaagaaatgcataaacttttgccattctcaccggattcagtcgtcactcatggtgatttctcacttgataaccttatttttgacgaggggaaattaataggttgtattgatgttggacgagtcggaatcgcagaccgataccaggatcttgccatcctatggaactgcctcggtgagttttctccttcattacagaaacggctttttcaaaaatatggtattgataatcctgatatgaataaattgcagtttcatttgatgctcgatgagtttttctaagaattaattcatgagcggatacatatttgaatgtatttagaaaaataaacaaataggggttccgcgcacatttccccgaaaagtgccacctgaaattgtaaacgttaatattttgttaaaattcgcgttaaatttttgttaaatcagctcattttttaaccaataggccgaaatcggcaaaatcccttataaatcaaaagaatagaccgagatagggttgagtgttgttccagtttggaacaagagtccactattaaagaacgtggactccaacgtcaaagggcgaaaaaccgtctatcagggcgatggcccactacgtgaaccatcaccctaatcaagttttttggggtcgaggtgccgtaaagcactaaatcggaaccctaaagggagcccccgatttagagcttgacggggaaagccggcgaacgtggcgagaaaggaagggaagaaagcgaaaggagcgggcgctagggcgctggcaagtgtagcggtcacgctgcgcgtaaccaccacacccgccgcgcttaatgcgccgctacagggcgcgtcccattcgcca

SEQ ID NO: 6 - DNA, 3063 bp, synthetic construct
  source 1..3063: mol_type = other DNA
atgagaggatcgcaccaccaccaccaccacccgattatggatgcgctgaaagaggcgaagctggaggcgaaggacctggacgaagttctgctggttggcggtagcacccgtattccggcggtgcagaccatgattgagcacaccctgggcaagaaaccgaaccgtagcattaacccggacgaagtggttgcgatcggtgcggcgattcaaggtggcgttctggcgggcgagattaacgatgtgctgctgctggacgttaccccgctgaccctgggtatcgaaaccctgggtggcattgcgaccccgctgattccgcgtaacaccaccattccggtgaccaaaagccagattttcagcaccgcggaaaacaaccaaaccgaggttaccatcagcgtggttcaaggcgagcgtcagctggcggcggacaacaagctgctgggtcgtttcaacctgagcggcattgagcaagcgccgcgtggtgtgccgcagatcgaagttagctttagcatcgacgtgaacggcattaccaccgttagcgcgaaagataagaaaaccaacaaggaacagaccatcaccattaagaacaccaccagcctgagcgaggaagagatcgaacgtatggtgaaagaggcggaagagaaccgtgaggcggatgcgaagaaaaaggaaaagattgaggttaccgtgcgtgcggaagcgctgatcaaccaactggaaaagagcctggaggaccagggtgataaagtggacgcgaagcaaaaagaaaccctggagaaacagatccaagagctgaaggacctggttaaggaagagaaaattgaagagctgaagaccaaactggatcagatcgaacaagcggcgcaggcgtttgcgcaggcggcggcgcagcaagcgaacaccagcgacaccagcagcgacgatcaaccgattgaagcggaagtgaaagaaaacgaggcggcggcgaaagaagcggcggcgaaagaggcggcggcgaaaggtaccggtcagccgaccaccatcaagttcgcgaccagccaaggtagctattggccgatgatgctgggcatgaaggagatcatcaagatttacaacgaacagcataaaaacgacgcggattttatcccggtggagctgctgaccagcgacgttacccacaaaaacagcgagggtcagctgctgagcagcctggacagcgatctgagcaccaagcaaagcagcgattggaacctgatcctgggcaacaaggcgaccgcgtatgtggcgaacagctacgataaactgctggacgtgggcaccagcaccgttaacccgaacagctttccgaccaaaatcattaacaactataacaagctgctgggtgttgagggccagaccaccctgaagagcctgccgtacaacatcaacgacaccgatggtattgtgttcaacctggatatcatgaaggttctgttcgacatcatcaagcagggtggtggcaccattgacgagaacagcatcattgcgaaaaaggtgaaggaagcggagggtaaaggcaaccacatcccgagcagcagcatgttcagcgcgatcaagattaaagaaagcagcaaaaacaccggtttcagcggctataccgttaacgatagcacctttagcgacatcaaaaaggcgttcgagtttgcgcagaagatttacgataacaccgaaatcgacaccaccaagctgagcaaagatgtgaaagatgaggctgctgctaaagaggcggctgctaaagaagcggctgcgaagggatccagctttgttgcgtgcggcaccaccgcgaccggcctgagccagaccaaagaccacgcggtgaccaacgagagcattcgtgttgcgctgaccgacccggataacccgcgttggatcaacgcgcaaaaggatatcctgaactacatcgacaagaccgaaggtgcgatcagcaccattaccaaagatcaaaacgcgcagaacaactggctgacccagcaagcgaacctgaacccggcgccgaagggtttcatcattgcgccggagaacggcggtggcgtgggcaccgcggttaacagcattgcggagaagaacatcccgattgtggcgtacgaccgtctgatcaccggcagcaccagctacgattggtacgttagctacgacaacgaaaaggttggcgagctgcaaggcctgagcctggcggcgggtctgctgggtaaaaccgatggtgcgtttaaggacgaaaccgagatgctgaactatctgaaggatcacatgccgcaagaaaccgtgagcttctacgcggttgcgggtagccaagacgataacaacagccagtacttttataacggcgcgatgaagatcctgaaaaagctgatggaaaacagcaacggcaaagtggttgacctgagcccgcgtggtaacgcggtttatgtgccgggctggaactacggtgatgcgggccagcgtattcagcaattctttacccaatatcgtgacagcagcgtgccgaacggtgtgctgccggttacctacgataacgtgaccatcccgaaaagcgttctgaagggtttcctggcgccgaacgatggtatggcggagcaggcggttgacaagctgaaagcgaccaactacgatgtgcaaaaggttttcatcaccggtcaggattacaacgacaccgcgaaaaagctgatcaagaacggcgagcagaacatgaccatttacaaaccggacgttatcctgggcaaggttgcggtggaagttctgaaaaccctgattaacaaaaagaaagcgaacgcgaccgcgaccaaagaagacgtggagaacgcgctgaaaaacaacgaaaacaccaaggatatccacttccgttatgacgataccacctacaaagcgggtagcgttggcgcgtacaaaaacatcaaggcgattctggtgaacccggtggttgtgaccaagcagaacgttgacaacccgctggcgaacgcgcagcaaagcaccagcgcgaatgttagcgttagcgcgagcggcaccgttccgaccaatggcgtgacccagcatcatcatcatcatcattaa

SEQ ID NO: 7 - protein, 1020 aa, synthetic construct
MRGSHHHHHHPIMDALKEAKLEAKDLDEVLLVGGSTRIPAVQTMIEHTLGKKPNRSINPDEVVAIGAAIQGGVLAGEINDVLLLDVTPLTLGIETLGGIATPLIPRNTTIPVTKSQIFSTAENNQTEVTISVVQGERQLAADNKLLGRFNLSGIEQAPRGVPQIEVSFSIDVNGITTVSAKDKKTNKEQTITIKNTTSLSEEEIERMVKEAEENREADAKKKEKIEVTVRAEALINQLEKSLEDQGDKVDAKQKETLEKQIQELKDLVKEEKIEELKTKLDQIEQAAQAFAQAAAQQANTSDTSSDDQPIEAEVKENEAAAKEAAAKEAAAKGTGQPTTIKFATSQGSYWPMMLGMKEIIKIYNEQHKNDADFIPVELLTSDVTHKNSEGQLLSSLDSDLSTKQSSDWNLILGNKATAYVANSYDKLLDVGTSTVNPNSFPTKIINNYNKLLGVEGQTTLKSLPYNINDTDGIVFNLDIMKVLFDIIKQGGGTIDENSIIAKKVKEAEGKGNHIPSSSMFSAIKIKESSKNTGFSGYTVNDSTFSDIKKAFEFAQKIYDNTEIDTTKLSKDVKDEAAAKEAAAKEAAAKGSSFVACGTTATGLSQTKDHAVTNESIRVALTDPDNPRWINAQKDILNYIDKTEGAISTITKDQNAQNNWLTQQANLNPAPKGFIIAPENGGGVGTAVNSIAEKNIPIVAYDRLITGSTSYDWYVSYDNEKVGELQGLSLAAGLLGKTDGAFKDETEMLNYLKDHMPQETVSFYAVAGSQDDNNSQYFYNGAMKILKKLMENSNGKVVDLSPRGNAVYVPGWNYGDAGQRIQQFFTQYRDSSVPNGVLPVTYDNVTIPKSVLKGFLAPNDGMAEQAVDKLKATNYDVQKVFITGQDYNDTAKKLIKNGEQNMTIYKPDVILGKVAVEVLKTLINKKKANATATKEDVENALKNNENTKDIHFRYDDTTYKAGSVGAYKNIKAILVNPVVVTKQNVDNPLANAQQSTSANVSVSASGTVPTNGVTQHHHHHH

SEQ ID NO: 8 - DNA, 996 bp, synthetic construct
  source 1..996: mol_type = other DNA
atgagaggatcgcaccaccaccaccaccacccgattatggatgcgctgaaagaggcgaagctggaggcgaaggacctggacgaagttctgctggttggcggtagcacccgtattccggcggtgcagaccatgattgagcacaccctgggcaagaaaccgaaccgtagcattaacccggacgaagtggttgcgatcggtgcggcgattcaaggtggcgttctggcgggcgagattaacgatgtgctgctgctggacgttaccccgctgaccctgggtatcgaaaccctgggtggcattgcgaccccgctgattccgcgtaacaccaccattccggtgaccaaaagccagattttcagcaccgcggaaaacaaccaaaccgaggttaccatcagcgtggttcaaggcgagcgtcagctggcggcggacaacaagctgctgggtcgtttcaacctgagcggcattgagcaagcgccgcgtggtgtgccgcagatcgaagttagctttagcatcgacgtgaacggcattaccaccgttagcgcgaaagataagaaaaccaacaaggaacagaccatcaccattaagaacaccaccagcctgagcgaggaagagatcgaacgtatggtgaaagaggcggaagagaaccgtgaggcggatgcgaagaaaaaggaaaagattgaggttaccgtgcgtgcggaagcgctgatcaaccaactggaaaagagcctggaggaccagggtgataaagtggacgcgaagcaaaaagaaaccctggagaaacagatccaagagctgaaggacctggttaaggaagagaaaattgaagagctgaagaccaaactggatcagatcgaacaagcggcgcaggcgtttgcgcaggcggcggcgcagcaagcgaacaccagcgacaccagcagcgacgatcaaccgattgaagcggaagtgaaagaaaacgaggcggcggcgaaagaagcggcggcgaaagaggcggcggcgaaa

SEQ ID NO: 9 - protein, 332 aa, synthetic construct
MRGSHHHHHHPIMDALKEAKLEAKDLDEVLLVGGSTRIPAVQTMIEHTLGKKPNRSINPDEVVAIGAAIQGGVLAGEINDVLLLDVTPLTLGIETLGGIATPLIPRNTTIPVTKSQIFSTAENNQTEVTISVVQGERQLAADNKLLGRFNLSGIEQAPRGVPQIEVSFSIDVNGITTVSAKDKKTNKEQTITIKNTTSLSEEEIERMVKEAEENREADAKKKEKIEVTVRAEALINQLEKSLEDQGDKVDAKQKETLEKQIQELKDLVKEEKIEELKTKLDQIEQAAQAFAQAAAQQANTSDTSSDDQPIEAEVKENEAAAKEAAAKEAAAK

SEQ ID NO: 10 - DNA, 765 bp, synthetic construct
  source 1..765: mol_type = other DNA
ggtcagccgaccaccatcaagttcgcgaccagccaaggtagctattggccgatgatgctgggcatgaaggagatcatcaagatttacaacgaacagcataaaaacgacgcggattttatcccggtggagctgctgaccagcgacgttacccacaaaaacagcgagggtcagctgctgagcagcctggacagcgatctgagcaccaagcaaagcagcgattggaacctgatcctgggcaacaaggcgaccgcgtatgtggcgaacagctacgataaactgctggacgtgggcaccagcaccgttaacccgaacagctttccgaccaaaatcattaacaactataacaagctgctgggtgttgagggccagaccaccctgaagagcctgccgtacaacatcaacgacaccgatggtattgtgttcaacctggatatcatgaaggttctgttcgacatcatcaagcagggtggtggcaccattgacgagaacagcatcattgcgaaaaaggtgaaggaagcggagggtaaaggcaaccacatcccgagcagcagcatgttcagcgcgatcaagattaaagaaagcagcaaaaacaccggtttcagcggctataccgttaacgatagcacctttagcgacatcaaaaaggcgttcgagtttgcgcagaagatttacgataacaccgaaatcgacaccaccaagctgagcaaagatgtgaaagatgaggctgctgctaaagaggcggctgctaaagaagcggctgcgaag

SEQ ID NO: 11 - protein, 255 aa, synthetic construct
GQPTTIKFATSQGSYWPMMLGMKEIIKIYNEQHKNDADFIPVELLTSDVTHKNSEGQLLSSLDSDLSTKQSSDWNLILGNKATAYVANSYDKLLDVGTSTVNPNSFPTKIINNYNKLLGVEGQTTLKSLPYNINDTDGIVFNLDIMKVLFDIIKQGGGTIDENSIIAKKVKEAEGKGNHIPSSSMFSAIKIKESSKNTGFSGYTVNDSTFSDIKKAFEFAQKIYDNTEIDTTKLSKDVKDEAAAKEAAAKEAAAK

SEQ ID NO: 12 - DNA, 1287 bp, synthetic construct
  source 1..1287: mol_type = other DNA
agctttgttgcgtgcggcaccaccgcgaccggcctgagccagaccaaagaccacgcggtgaccaacgagagcattcgtgttgcgctgaccgacccggataacccgcgttggatcaacgcgcaaaaggatatcctgaactacatcgacaagaccgaaggtgcgatcagcaccattaccaaagatcaaaacgcgcagaacaactggctgacccagcaagcgaacctgaacccggcgccgaagggtttcatcattgcgccggagaacggcggtggcgtgggcaccgcggttaacagcattgcggagaagaacatcccgattgtggcgtacgaccgtctgatcaccggcagcaccagctacgattggtacgttagctacgacaacgaaaaggttggcgagctgcaaggcctgagcctggcggcgggtctgctgggtaaaaccgatggtgcgtttaaggacgaaaccgagatgctgaactatctgaaggatcacatgccgcaagaaaccgtgagcttctacgcggttgcgggtagccaagacgataacaacagccagtacttttataacggcgcgatgaagatcctgaaaaagctgatggaaaacagcaacggcaaagtggttgacctgagcccgcgtggtaacgcggtttatgtgccgggctggaactacggtgatgcgggccagcgtattcagcaattctttacccaatatcgtgacagcagcgtgccgaacggtgtgctgccggttacctacgataacgtgaccatcccgaaaagcgttctgaagggtttcctggcgccgaacgatggtatggcggagcaggcggttgacaagctgaaagcgaccaactacgatgtgcaaaaggttttcatcaccggtcaggattacaacgacaccgcgaaaaagctgatcaagaacggcgagcagaacatgaccatttacaaaccggacgttatcctgggcaaggttgcggtggaagttctgaaaaccctgattaacaaaaagaaagcgaacgcgaccgcgaccaaagaagacgtggagaacgcgctgaaaaacaacgaaaacaccaaggatatccacttccgttatgacgataccacctacaaagcgggtagcgttggcgcgtacaaaaacatcaaggcgattctggtgaacccggtggttgtgaccaagcagaacgttgacaacccgctggcgaacgcgcagcaaagcaccagcgcgaatgttagcgttagcgcgagcggcaccgttccgaccaatggcgtgacccagcatcatcatcatcatcat

SEQ ID NO: 13 - protein, 429 aa, synthetic construct
SFVACGTTATGLSQTKDHAVTNESIRVALTDPDNPRWINAQKDILNYIDKTEGAISTITKDQNAQNNWLTQQANLNPAPKGFIIAPENGGGVGTAVNSIAEKNIPIVAYDRLITGSTSYDWYVSYDNEKVGELQGLSLAAGLLGKTDGAFKDETEMLNYLKDHMPQETVSFYAVAGSQDDNNSQYFYNGAMKILKKLMENSNGKVVDLSPRGNAVYVPGWNYGDAGQRIQQFFTQYRDSSVPNGVLPVTYDNVTIPKSVLKGFLAPNDGMAEQAVDKLKATNYDVQKVFITGQDYNDTAKKLIKNGEQNMTIYKPDVILGKVAVEVLKTLINKKKANATATKEDVENALKNNENTKDIHFRYDDTTYKAGSVGAYKNIKAILVNPVVVTKQNVDNPLANAQQSTSANVSVSASGTVPTNGVTQHHHHHH